European Patent Application EP 4 386 082 A1, published June 19, 2024. Title: A method for producing a pluripotent stem cell. Applicant: KANEKA CORPORATION. The sequence listing filed with the application follows.

SEQUENCE LISTING (14 sequences)

SEQ ID NO: 1 - DNA, 21 bp, synthetic construct
  misc_feature 1..21: note = Synthetic DNA
  source 1..21: mol_type = other DNA
cctcatgaagatcctcaccga

SEQ ID NO: 2 - DNA, 21 bp, synthetic construct
  misc_feature 1..21: note = Synthetic DNA
  source 1..21: mol_type = other DNA
ttgccaatggtgatgacctgg

SEQ ID NO: 3 - DNA, 23 bp, synthetic construct
  misc_feature 1..23: note = Synthetic DNA
  source 1..23: mol_type = other DNA
agtgggtggaggaagctgacaac

SEQ ID NO: 4 - DNA, 24 bp, synthetic construct
  misc_feature 1..24: note = Synthetic DNA
  source 1..24: mol_type = other DNA
tcgttgtgcatagtcgctgcttga

SEQ ID NO: 5 - DNA, 22 bp, synthetic construct
  misc_feature 1..22: note = Synthetic DNA
  source 1..22: mol_type = other DNA
caccaatcccatccacactcac

SEQ ID NO: 6 - DNA, 21 bp, synthetic construct
  misc_feature 1..21: note = Synthetic DNA
  source 1..21: mol_type = other DNA
gcaaagctcctaccgtaccac

SEQ ID NO: 7 - DNA, 24 bp, synthetic construct
  misc_feature 1..24: note = Synthetic DNA
  source 1..24: mol_type = other DNA
agcctccagcagatgcaagaactc

SEQ ID NO: 8 - DNA, 24 bp, synthetic construct
  misc_feature 1..24: note = Synthetic DNA
  source 1..24: mol_type = other DNA
ttgctccacattggaaggttccca

SEQ ID NO: 9 - DNA, 23 bp, synthetic construct
  misc_feature 1..23: note = Synthetic DNA
  source 1..23: mol_type = other DNA
tcacaaagagatgatggaggaac

SEQ ID NO: 10 - DNA, 20 bp, synthetic construct
  misc_feature 1..20: note = Synthetic DNA
  source 1..20: mol_type = other DNA
acatgcaggtgagttgtcag

SEQ ID NO: 11 - DNA, 20 bp, synthetic construct
  misc_feature 1..20: note = Synthetic DNA
  source 1..20: mol_type = other DNA
atctgcacttcgtgtgcaag

SEQ ID NO: 12 - DNA, 23 bp, synthetic construct
  misc_feature 1..23: note = Synthetic DNA
  source 1..23: mol_type = other DNA
gagtctgaggatttccttagctc

SEQ ID NO: 13 - DNA, 21 bp, synthetic construct
  misc_feature 1..21: note = Synthetic DNA
  source 1..21: mol_type = other DNA
aggaatggacttgaaacaagg

SEQ ID NO: 14 - DNA, 20 bp, synthetic construct
  misc_feature 1..20: note = Synthetic DNA
  source 1..20: mol_type = other DNA
gcaaagcttgttgatcatgg